European Patent Specification EP 3 908 308 B1, published July 22, 2026. Title: SMALL MOLECULE ANALOGS OF THE PROTEIN E4ORF1 IN THE TREATMENT AND PREVENTION OF DIABETES. Applicant: Texas Tech University System. The sequence listing filed with the application follows.

SEQUENCE LISTING (1 sequence)

SEQ ID NO: 1 - protein, 125 aa, Artificial Sequence
  Ad36 E4orf1 Protein Translation
MAESLYAFIDSPGGIAPVQEGASNRYIFFCPESFHIPPHGVILLHLRVSVLVPTGYQGRFMALNDYHARGILTQSDVIFAGRRHDLSVLLFNHTDRFLYVREGHPVGTLLLERVIFPSVRIATLV